European Patent Specification EP 4 006 155 B1, published September 17, 2025. Title: Detection method or quantitative method of SMN1 genes. Applicant: SEKISUI MEDICAL CO., LTD. The sequence listing filed with the application follows.

SEQUENCE LISTING (23 sequences)

SEQ ID NO: 1 - DNA, 30 bp, Artificial Sequence
  primer
taacttcctttattttccttacagggtttc

SEQ ID NO: 2 - DNA, 29 bp, Artificial Sequence
  primer
aacttcctttattttccttacagggtttc

SEQ ID NO: 3 - DNA, 28 bp, Artificial Sequence
  primer
acttcctttattttccttacagggtttc

SEQ ID NO: 4 - DNA, 27 bp, Artificial Sequence
  primer
cttcctttattttccttacagggtttc

SEQ ID NO: 5 - DNA, 26 bp, Artificial Sequence
  primer
ttcctttattttccttacagggtttc

SEQ ID NO: 6 - DNA, 25 bp, Artificial Sequence
  primer
tcctttattttccttacagggtttc

SEQ ID NO: 7 - DNA, 24 bp, Artificial Sequence
  primer
cctttattttccttacagggtttc

SEQ ID NO: 8 - DNA, 23 bp, Artificial Sequence
  primer
ctttattttccttacagggtttc

SEQ ID NO: 9 - DNA, 22 bp, Artificial Sequence
  primer
tttattttccttacagggtttc

SEQ ID NO: 10 - DNA, 26 bp, Artificial Sequence
  primer
cactttcataatgctggcagacttac

SEQ ID NO: 11 - DNA, 400 bp, Homo sapiens
caacttaatttctgatcatattttgttgaataaaataagtaaaatgtcttgtgaaacaaaatgctttttaacatccatataaagctatctatatatagctatctatgtctatatagctattttttttaacttcctttattttccttacagggtttcagacaaaatcaaaaagaaggaaggtgctcacattccttaaattaaggagtaagtctgccagcattatgaaagtgaatcttacttttgtaaaactttatggtttgtggaaaacaaatgtttttgaacatttaaaaagttcagatgttaaaaagttgaaaggttaatgtaaaacaatcaatattaaagaattttgatgccaaaactattagataaaaggttaatctacatccctactagaattctc

SEQ ID NO: 12 - DNA, 400 bp, Homo sapiens
caacttaatttctgatcatattttgttgaataaaataagtaaaatgtcttgtgaaacaaaatgctttttaacatccatataaagctatctatatatagctatctatatctatatagctattttttttaacttcctttattttccttacagggttttagacaaaatcaaaaagaaggaaggtgctcacattccttaaattaaggagtaagtctgccagcattatgaaagtgaatcttacttttgtaaaactttatggtttgtggaaaacaaatgtttttgaacatttaaaaagttcagatgttagaaagttgaaaggttaatgtaaaacaatcaatattaaagaattttgatgccaaaactattagataaaaggttaatctacatccctactagaattctc

SEQ ID NO: 13 - DNA, 28 bp, Artificial Sequence
  primer
agtaaaatgtcttgtgaaacaaaatgct

SEQ ID NO: 14 - DNA, 27 bp, Artificial Sequence
  primer
caccttccttctttttgattttgtctg

SEQ ID NO: 15 - DNA, 26 bp, Artificial Sequence
  primer
accttccttctttttgattttgtctg

SEQ ID NO: 16 - DNA, 25 bp, Artificial Sequence
  primer
ccttccttctttttgattttgtctg

SEQ ID NO: 17 - DNA, 24 bp, Artificial Sequence
  primer
cttccttctttttgattttgtctg

SEQ ID NO: 18 - DNA, 23 bp, Artificial Sequence
  primer
ttccttctttttgattttgtctg

SEQ ID NO: 19 - DNA, 22 bp, Artificial Sequence
  primer
tccttctttttgattttgtctg

SEQ ID NO: 20 - DNA, 21 bp, Artificial Sequence
  primer
ccttctttttgattttgtctg

SEQ ID NO: 21 - DNA, 20 bp, Artificial Sequence
  primer
cttctttttgattttgtctg

SEQ ID NO: 22 - DNA, 19 bp, Artificial Sequence
  primer
ttctttttgattttgtctg

SEQ ID NO: 23 - DNA, 30 bp, Artificial Sequence
  probe
ggaaggtgctcacattccttaaattaagga